European Patent Specification EP 4 086 343 B1, published August 19, 2026. Title: USE OF BIOLOGICAL ENZYME FOR PREPARING ORLISTAT INTERMEDIATE, AND PREPARATION METHOD. Applicant: ZEIN BIOTECHNOLOGY CO.,LTD. The sequence listing filed with the application follows.

SEQUENCE LISTING (9 sequences)

SEQ ID NO: 1 - protein, 249 aa, Artificial Sequence
  Amino acid sequence of the ketoreductase
MGKLDNKVAVITGGNSGMGLATAQRFVSEGAYVFITGRRQAELDKAVDLIGKNVTGVQGDVSNLADLDRLYATVKEQKGRVDVLFANAGVGELAPLGSITEEQFDKVFNINVRGLLFTVQKALPLFQDGGSIILNASIASIKGMPAFSVYSASKAAVRSFARSWTVDLKGRKIRINTLSPGPIDTPILSGLASTEEELKQVKADLAAQVPLGRMGTSDEIANVALFLASDDSSYVTGIELFVDGGMAQI

SEQ ID NO: 2 - protein, 259 aa, Artificial Sequence
  Amino acid sequence of the ketoreductase
MARLAGKVALVTGGASVPGLGSATAIRFAQEGATVYLTDRDLAGAQAVAAQITAAGGRATALEHDVTSEADWDRVLAAIDAAEGRLDILVNNAGIAVLGPLEDVTAADFLRQNDVNLNSVFHGSKRALVMMRRPGDGGTARGGSIINISSVAGLIGVPGCGSYAASKGGVRLFSKVVALEGAADGVRCNSVHPGMIATNIQGVALEDNAANFDAVMALIPMVRMGEPEDIANMNLFLASDESRYITGAEFVVDGGMTAR

SEQ ID NO: 3 - protein, 263 aa, Artificial Sequence
  Amino acid sequence of the glucose dehydrogenase
MYMYPDLKGKVVAITGAASGLGKAMAIRFGKEQAKVVINYYSNKQDPNEVKEEVIKAGGEAVVVQGDVTKEEDVKNIVQTAIKEFGTLDIMINNAGLENPVPSHEMPLKDWDKVIGTNLTGAFLGSREAIKYFVENDIKGNVINMSSVHEVIPWPLFVHYAASKGGIKLMTETLALEYAPKGIRVNNIGPGAINTPINAEKFADPKQKADVESMIPMGYIGEPEEIAAVAAWLASKEASYVTGITLFADGGMTQYPSFQAGRG

SEQ ID NO: 4 - protein, 248 aa, Artificial Sequence
  Amino acid sequence of the ketoreductase
MSSPAPTVYVISGASRGIGFAITSILAQHDNVLIFAGARDLKSAQLNELAQKSSGKVIPVKLESTSVEDAAALAKVVEEKAGKVDYVLAVAGISQSTDPIAQVSLDDVRRHFEVNTIGPLVLFQALLPLTTKSTAPHFIVVSTIAGSIASMPQVTFPVSAYAISKTAVNSAVGRIAIEHPDLDAFVCHPGFVSSDMVKQFAEKTGAPLSDFESFGMITPEESAASLVKLFDEAKKETHSGKFFNVDGT

SEQ ID NO: 5 - protein, 77 aa, Artificial Sequence
  Amino acid sequence of the linker
EFEEEEKKKQQEEEAERLRRIQEEMEKERKRREEDEERRRKEEEERRMKLEMEAKRKQEEEERKKREDDEKRKKKKL

SEQ ID NO: 6 - DNA, 1767 bp, Artificial Sequence
  Nucleotide sequence of the fusion enzyme
atgtatatgtatccggatttaaaaggaaaagtcgtcgctattacaggagctgcttcagggctcggaaaggcgatggccattcgcttcggcaaggagcaggcaaaagtggttatcaactattatagtaataaacaagatccgaacgaggtaaaagaagaggtcatcaaggcgggcggtgaagctgttgtcgtccaaggagatgtcacgaaagaggaagatgtaaaaaatatcgtgcaaacggcaattaaggagttcggcacactcgatattatgattaataatgccggtcttgaaaatcctgtgccatctcacgaaatgccgctcaaggattgggataaagtcatcggcacgaacttaacgggtgcctttttaggaagccgtgaagcgattaaatatttcgtagaaaacgatattaagggaaatgtcattaacatgtccagtgtgcacgaagtgattccttggccgttatttgtccactatgcggcaagtaaaggcgggataaagctgatgacagaaacattagcgttggaatacgcgccgaagggcattcgcgtcaataatattgggccaggtgcgatcaacacgccaatcaatgctgaaaaattcgctgaccctaaacagaaagctgatgtagaaagcatgattccaatgggatatatcggcgaaccggaggagatcgccgcagtagcagcctggcttgcttcgaaggaagccagctacgtcacaggcatcacgttattcgcggacggcggtatgacacaatatccttcattccaggcaggccgcggtgaattcgaagaagaggaaaaaaagaaacagcaggaagaagaagcggaacgtctgcgtcgtattcaggaggagatggagaaagaacgtaaacgccgcgaagaggacgaagaacgccgtcgtaaagaggaagaggagcgccgtatgaaactggaaatggaagcgaaacgcaaacaagaggaggaagagcgtaaaaagcgcgaggatgatgaaaaacgtaagaaaaaaaagcttatgtcttcgcctgctcccaccgtctacgtcatctctggcgcctctcgcggcatcggcttcgccatcacctccattctcgctcaacacgacaacgtattgatctttgccggcgcacgcgacctcaagtcggcgcaactgaacgagctcgctcagaagtctagcggcaaggtcatcccggtcaagctcgagtcgacgagtgtcgaggatgccgctgcgcttgccaaggtcgtcgaggagaaggctggaaaggtggactacgtcttggccgtcgccggcatctcccagtcgaccgaccccatcgcccaagtctccctcgacgacgtcaggcgtcacttcgaggtcaacaccatcggccctctcgtcctcttccaggcgctcctccccctcaccaccaagtcgaccgcgccgcacttcatcgtcgtctccaccatcgccggctcaatcgcctccatgcctcaagtcacgttccccgtgagcgcctacgctatctcgaagactgccgtcaactcggccgtaggacgaatcgcgatcgagcaccccgacctcgacgccttcgtctgccatccgggctttgtgagcagcgacatggtcaaacaatttgcggagaagacgggcgcaccgttgtcggactttgagtcgtttggcatgatcacccccgaagaatcggctgcgagtctcgttaagctgttcgacgaggccaagaaggagacgcactcgggcaagttctttaacgtcgacgggacctag

SEQ ID NO: 7 - DNA, 1779 bp, Artificial Sequence
  Nucleotide sequence of the fusion enzyme
atgtcttcgcctgctcccaccgtctacgtcatctctggcgcctctcgcggcatcggcttcgccatcacctccattctcgctcaacacgacaacgtattgatctttgccggcgcacgcgacctcaagtcggcgcaactgaacgagctcgctcagaagtctagcggcaaggtcatcccggtcaagctcgagtcgacgagtgtcgaggatgccgctgcgcttgccaaggtcgtcgaggagaaggctggaaaggtggactacgtcttggccgtcgccggcatctcccagtcgaccgaccccatcgcccaagtctccctcgacgacgtcaggcgtcacttcgaggtcaacaccatcggccctctcgtcctcttccaggcgctcctccccctcaccaccaagtcgaccgcgccgcacttcatcgtcgtctccaccatcgccggctcaatcgcctccatgcctcaagtcacgttccccgtgagcgcctacgctatctcgaagactgccgtcaactcggccgtaggacgaatcgcgatcgagcaccccgacctcgacgccttcgtctgccatccgggctttgtgagcagcgacatggtcaaacaatttgcggagaagacgggcgcaccgttgtcggactttgagtcgtttggcatgatcacccccgaagaatcggctgcgagtctcgttaagctgttcgacgaggccaagaaggagacgcactcgggcaagttctttaacgtcgacgggaccgaattcgaagaagaggaaaaaaagaaacagcaggaagaagaagcggaacgtctgcgtcgtattcaggaggagatggagaaagaacgtaaacgccgcgaagaggacgaagaacgccgtcgtaaagaggaagaggagcgccgtatgaaactggaaatggaagcgaaacgcaaacaagaggaggaagagcgtaaaaagcgcgaggatgatgaaaaacgtaagaaaaaaaagcttatgtatccggatttaaaaggaaaagtcgtcgctattacaggagctgcttcagggctcggaaaggcgatggccattcgcttcggcaaggagcaggcaaaagtggttatcaactattatagtaataaacaagatccgaacgaggtaaaagaagaggtcatcaaggcgggcggtgaagctgttgtcgtccaaggagatgtcacgaaagaggaagatgtaaaaaatatcgtgcaaacggcaattaaggagttcggcacactcgatattatgattaataatgccggtcttgaaaatcctgtgccatctcacgaaatgccgctcaaggattgggataaagtcatcggcacgaacttaacgggtgcctttttaggaagccgtgaagcgattaaatatttcgtagaaaacgatattaagggaaatgtcattaacatgtccagtgtgcacgaagtgattccttggccgttatttgtccactatgcggcaagtaaaggcgggataaagctgatgacagaaacattagcgttggaatacgcgccgaagggcattcgcgtcaataatattgggccaggtgcgatcaacacgccaatcaatgctgaaaaattcgctgaccctaaacagaaagctgatgtagaaagcatgattccaatgggatatatcggcgaaccggaggagatcgccgcagtagcagcctggcttgcttcgaaggaagccagctacgtcacaggcatcacgttattcgcggacggcggtatgacacaatatccttcattccaggcaggccgcggtcaccaccaccaccaccactag

SEQ ID NO: 8 - protein, 588 aa, Artificial Sequence
  Amino acid sequence of the fusion enzyme
MYMYPDLKGKVVAITGAASGLGKAMAIRFGKEQAKVVINYYSNKQDPNEVKEEVIKAGGEAVVVQGDVTKEEDVKNIVQTAIKEFGTLDIMINNAGLENPVPSHEMPLKDWDKVIGTNLTGAFLGSREAIKYFVENDIKGNVINMSSVHEVIPWPLFVHYAASKGGIKLMTETLALEYAPKGIRVNNIGPGAINTPINAEKFADPKQKADVESMIPMGYIGEPEEIAAVAAWLASKEASYVTGITLFADGGMTQYPSFQAGRGEFEEEEKKKQQEEEAERLRRIQEEMEKERKRREEDEERRRKEEEERRMKLEMEAKRKQEEEERKKREDDEKRKKKKLMSSPAPTVYVISGASRGIGFAITSILAQHDNVLIFAGARDLKSAQLNELAQKSSGKVIPVKLESTSVEDAAALAKVVEEKAGKVDYVLAVAGISQSTDPIAQVSLDDVRRHFEVNTIGPLVLFQALLPLTTKSTAPHFIVVSTIAGSIASMPQVTFPVSAYAISKTAVNSAVGRIAIEHPDLDAFVCHPGFVSSDMVKQFAEKTGAPLSDFESFGMITPEESAASLVKLFDEAKKETHSGKFFNVDGT

SEQ ID NO: 9 - protein, 592 aa, Artificial Sequence
  Amino acid sequence of the fusion enzyme
MSSPAPTVYVISGASRGIGFAITSILAQHDNVLIFAGARDLKSAQLNELAQKSSGKVIPVKLESTSVEDAAALAKVVEEKAGKVDYVLAVAGISQSTDPIAQVSLDDVRRHFEVNTIGPLVLFQALLPLTTKSTAPHFIVVSTIAGSIASMPQVTFPVSAYAISKTAVNSAVGRIAIEHPDLDAFVCHPGFVSSDMVKQFAEKTGAPLSDFESFGMITPEESAASLVKLFDEAKKETHSGKFFNVDGTEFEEEEKKKQQEEEAERLRRIQEEMEKERKRREEDEERRRKEEEERRMKLEMEAKRKQEEEERKKREDDEKRKKKKLMYPDLKGKVVAITGAASGLGKAMAIRFGKEQAKVVINYYSNKQDPNEVKEEVIKAGGEAVVVQGDVTKEEDVKNIVQTAIKEFGTLDIMINNAGLENPVPSHEMPLKDWDKVIGTNLTGAFLGSREAIKYFVENDIKGNVINMSSVHEVIPWPLFVHYAASKGGIKLMTETLALEYAPKGIRVNNIGPGAINTPINAEKFADPKQKADVESMIPMGYIGEPEEIAAVAAWLASKEASYVTGITLFADGGMTQYPSFQAGRGHHHHHH